European Patent Application EP 4 450 618 A2, published October 23, 2024. Title: SOYBEANS HAVING HIGH GERMINATION RATES AND ULTRA-LOW RAFFINOSE AND STACHYOSE CONTENT. Applicant: Benson Hill Seeds, Inc. Application EP. The sequence listing filed with the application follows.

SEQUENCE LISTING (18 sequences)

SEQ ID NO: 1 - DNA, 2346 bp, Glycine max
  source 1..2346: mol_type = other DNA
atggctccaagcataagcaaaactgtggaactaaattcatttggtcttgtcaacggtaatttgcctttgtccataaccctagaaggatcaaatttcctcgccaacggccacccttttctcacggaagttcccgaaaacataatagtcaccccttcacccatcgacgccaagagtagtaagaacaacgaggacgacgacgtcgtaggttgcttcgtgggcttccacgcggacgagcccagaagccgacacgtggcttccctggggaagctcagaggaataaaattcatgagcatattccggtttaaggtgtggtggaccactcactgggtcggtagcaacggacacgaactggagcacgagacacagatgatgcttctcgacaaaaacgaccagctcggacgcccctttgtgttgattctcccgatcctccaagcctcgttccgagcctccctgcaacccggtttggatgattacgtggacgtttgcatggagagcgggtcgacacgtgtctgtggctccagcttcgggagctgcttatacgtccacgttggccatgacccgtatcagttgcttagagaagcaactaaagtcgttaggatgcatttggggacgttcaagcttctcgaggagaaaaccgcgccagtgatcatagacaagtttggttggtgtacatgggacgcgttttacttgaaggtgcatccctcaggtgtgtgggaaggggtgaaagggttggtggagggagggtgccctccagggatggtcctaatcgacgacgggtggcaagccatttgtcacgacgaggaccccataacggaccaagagggtatgaagcgaacctccgcaggggagcaaatgccatgcaggttggtgaagttggaggaaaattacaagttcagacagtattgtagtggaaaggattctgagaagggtatgggtgcctttgttagggacttgaaggaacagtttaggagcgtggagcaggtgtatgtgtggcacgcgctttgtgggtattggggtggggtcagacccaaggttccgggcatgccccaggctaaggttgtcactccgaagctgtccaatggactaaaattgacaatgaaggatttagcggtggataagatcgtcagtaacggagttggactggtgccaccacacctggctcaccttttgtacgaagggctccactcccgtttggaatctgcgggtattgacggtgttaaggttgacgttatacacttgctcgagatgctatccgaggaatacggtggccgtgttgagctagccaaagcttattacaaagcgctcactgcttcggtgaagaagcatttcaaaggcaatggggtcattgcgagcatggagcattgtaatgacttctttctccttggtaccgaagccatagcccttgggcgcgtaggagatgatttttggtgcactgatccctctggagatccaaatggcacgtattggctccaagggtgtcacatggtgcactgtgcctacaacagcttgtggatggggaattttattcagccggattgggacatgttccagtccactcacccttgtgccgaattccatgcagcctctagggccatctctggtggaccagtttacgttagtgattgtgttggaaagcacaacttcaagttgctcaagagcctcgctttgcctgatgggacgattttgcgttgtcaacactatgcactccccacacgagactgtttgtttgaagaccccttgcatgatgggaagacaatgctcaaaatttggaatctcaacaaatatacaggtgttttgggtctatttaattgccaaggaggtgggtggtgtcccgtaactaggagaaacaagagtgcctctgaattttcacaaactgtgacatgcttagcgagtcctcaagacattgaatggagcaatgggaaaagcccaatatgcataaaagggatgaatgtgtttgctgtatatttgttcaaggaccacaaactaaagctcatgaaggcatcagagaaattggaagtttcacttgagccatttacttttgagctattgacagtgtctccagtgattgtgctgtcaaaaaagttaattcaatttgctccaattggattagtgaacatgcttaacactggtggtgccattcagtccatggagtttgacaaccacatagatgtggtcaaaattggggttaggggttgtggggagatgaaggtgtttgcatcagagaaaccagttagttgcaaactagatggggtagttgtaaaatttgattatgaggataaaatgctgagagtgcaagttccctggcctagtgcttcaaaattgtcaatggttgagtttttattttga

SEQ ID NO: 2 - protein, 781 aa, Glycine max
MAPSISKTVELNSFGLVNGNLPLSITLEGSNFLANGHPFLTEVPENIIVTPSPIDAKSSKNNEDDDVVGCFVGFHADEPRSRHVASLGKLRGIKFMSIFRFKVWWTTHWVGSNGHELEHETQMMLLDKNDQLGRPFVLILPILQASFRASLQPGLDDYVDVCMESGSTRVCGSSFGSCLYVHVGHDPYQLLREATKVVRMHLGTFKLLEEKTAPVIIDKFGWCTWDAFYLKVHPSGVWEGVKGLVEGGCPPGMVLIDDGWQAICHDEDPITDQEGMKRTSAGEQMPCRLVKLEENYKFRQYCSGKDSEKGMGAFVRDLKEQFRSVEQVYVWHALCGYWGGVRPKVPGMPQAKVVTPKLSNGLKLTMKDLAVDKIVSNGVGLVPPHLAHLLYEGLHSRLESAGIDGVKVDVIHLLEMLSEEYGGRVELAKAYYKALTASVKKHFKGNGVIASMEHCNDFFLLGTEAIALGRVGDDFWCTDPSGDPNGTYWLQGCHMVHCAYNSLWMGNFIQPDWDMFQSTHPCAEFHAASRAISGGPVYVSDCVGKHNFKLLKSLALPDGTILRCQHYALPTRDCLFEDPLHDGKTMLKIWNLNKYTGVLGLFNCQGGGWCPVTRRNKSASEFSQTVTCLASPQDIEWSNGKSPICIKGMNVFAVYLFKDHKLKLMKASEKLEVSLEPFTFELLTVSPVIVLSKKLIQFAPIGLVNMLNTGGAIQSMEFDNHIDVVKIGVRGCGEMKVFASEKPVSCKLDGVVVKFDYEDKMLRVQVPWPSASKLSMVEFLF

SEQ ID NO: 3 - DNA, 2277 bp, Glycine max
  source 1..2277: mol_type = other DNA
atgggtccaagctcgaagaaagcttcagctaaatcaggtgtgacaaagcacatgaagggcttcagcctctgcaactcaaccctaaaagtaaatgggcaagtcatcctctcccaagtccccaagaacgtaaccctcaccccatgcacctacgacactcacaccaccggatgcttcctcggtttccacgccacctccccaaaatcccgccacgtggcacccttaggacagcttaaaaacataagcttcacttccatcttccggttcaaggtttggtggaccactctctggaccggctccaacggccgcgacctggaaaccgaaacccaattcctcatgctccaatcccacccttatgttctcttcctacccatcctccaacccccatttcgcgcctcgctgcagcctcactcagacgacaacgttgcggtgtgtgtggagagcggctccagccacgtaacagcctcatcattcgacactgtcgtctacttgcacgcaggggacaaccccttcacgctggtcaaggaagccatgcgcgtcgtccgggcccacttggggagcttcaagcttctggaagagaaaacagttccgggaatggtggacaagttcggttggtgcacgtgggacgccttttacctgacggtgcaccctgagggcgtcagagagggcgtgaagggcctggttgacggcggttgtcctccgggattcgtcctgatcgacgacggctggcagtgcatcagccacgattccgatccggagaaggaggggatgaatcagacggtggccggggagcaaatgccctgcaggttgattagttacgaggagaattacaagtttaggagctataaggaagggaaggggttgaaggggtttgtgagagaattgaaggaggagtttgggtcggtggagtacgtgtacgtgtggcacgcgctgtgcgggtattggggaggggtgaggccgggggtggcggggatggcggaggcggcggtggagaagccaaagctgacggaggggttgaagggaacgatggaggatctggcggtggacaagattgtgaataatggggtcggggtggtgccgccggagctggtgggggaaatgtatgagcgccttcacgcgcacttggagagtgcgggtattgatggggtcaaagttgatgtcatccacttgctagaaatggtgtgtgagaaatatggagggcgagtggatatggcgaaagcatattacaaagctctcactgcttccgtgagaaaacattttaagggcaacggcgtcattgccagcatggagcattgcaacgatttcatgttgctgggaactgaagcaatatcccttggtcgtgttggggatgatttctggtgcactgacccttatggtgatccaaatggtacattttggctacaagggtgtcacatggtgcattgtgcatacaacagcttgtggatgggcaatttcatccacccagattgggacatgttccaatctactcatccttgtgctgccttccatgctgcctcaagagccatatctggtggccccatttacatcagtgacacagttgggaaccacaactttgagctgcttaagaccttggccttgccagatgggtccatcctcagatgtgagcactatgcactcccaaccagggactgtctctttgctgaccctctccatgatggcaaaacaatgctcaagatatggaacctcaacaagtacactggagttcttggggtgtttaactgccagggaggaggttggttccgtgagattaggtccaacaaatgtgctgctgagttttctcatagggtatcaaccaagaccaatatcaaagacattgaatgggatagtggaaagaatccaatttccattgaaggggtgcaacttttcgcttcgtatttcagccaagccaagaaactcatcctctcagcaccatctgatgacagtgaagagatttccttggagccattcaatttcgagcttataacagtttcccctgtgactgtcttgcctggcaagtcagtgaagtttgctcctattggtttggtgaatatgctaaacactggtggagcagtccagtctttagcttttgatgagggtcagaatttggttgaagttggtttaagaggcactggggagatgagagtctatgcctcagagaaaccaagaacttgtagaattgatggcaaagaagttgattttgaatatgaagggtctatggtcaacattcaagtaccatggcctggttcttcaaaattgtccactgttcagtatgtattttaa

SEQ ID NO: 4 - protein, 758 aa, Glycine max
MGPSSKKASAKSGVTKHMKGFSLCNSTLKVNGQVILSQVPKNVTLTPCTYDTHTTGCFLGFHATSPKSRHVAPLGQLKNISFTSIFRFKVWWTTLWTGSNGRDLETETQFLMLQSHPYVLFLPILQPPFRASLQPHSDDNVAVCVESGSSHVTASSFDTVVYLHAGDNPFTLVKEAMRVVRAHLGSFKLLEEKTVPGMVDKFGWCTWDAFYLTVHPEGVREGVKGLVDGGCPPGFVLIDDGWQCISHDSDPEKEGMNQTVAGEQMPCRLISYEENYKFRSYKEGKGLKGFVRELKEEFGSVEYVYVWHALCGYWGGVRPGVAGMAEAAVEKPKLTEGLKGTMEDLAVDKIVNNGVGVVPPELVGEMYERLHAHLESAGIDGVKVDVIHLLEMVCEKYGGRVDMAKAYYKALTASVRKHFKGNGVIASMEHCNDFMLLGTEAISLGRVGDDFWCTDPYGDPNGTFWLQGCHMVHCAYNSLWMGNFIHPDWDMFQSTHPCAAFHAASRAISGGPIYISDTVGNHNFELLKTLALPDGSILRCEHYALPTRDCLFADPLHDGKTMLKIWNLNKYTGVLGVFNCQGGGWFREIRSNKCAAEFSHRVSTKTNIKDIEWDSGKNPISIEGVQLFASYFSQAKKLILSAPSDDSEEISLEPFNFELITVSPVTVLPGKSVKFAPIGLVNMLNTGGAVQSLAFDEGQNLVEVGLRGTGEMRVYASEKPRTCRIDGKEVDFEYEGSMVNIQVPWPGSSKLSTVQYVF

SEQ ID NO: 5 - DNA, 2358 bp, Glycine max
  misc_feature 1064: note = n is a, c, g, or t
  source 1..2358: mol_type = other DNA
atggcgccaagcctaaccgccaagcaagaagcggcgcttctcaacgcaaatccacacttatccataaaactccaatcctcaactttcttcgctaacaaccacccaatcctcacccaagtcccaccgaacataacaacaaccactccaccgccccacgatgcttccaccacccccgccggatgcttcgtcggtttctccgccgacgaggcacgcagccggcacgtgatctccctcggcaaactgaggggtatcagattcacgagcattttccgcttcaagctctggtggagcacccactggtccggcagcaacggccgcgacgtggagaacgaaacccaaatgatgatcctccaaaacgacgccgtcgagggccgaccctacgtcctcctcctcccactcctcgaaggacccttccgagcctcgctccaacccggcctccacgacgacgtggacatctgcatggagagcggctccgcacgtgtcaccaagtcacgcttccgaacctccgtctacatgcacgtgcacgacgatccttttactctaatcgacgaagcgctgaaagtaatccgagtctatctcggaacgtttaggttaatggaagagaaaaccgtgccggggattattgacaagttcgggtggtgcacgtgggacgcgttttaccttaacgtgcacccggagggggtgcgggaaggaattaagggcctggtggagggagggtgtcctccggggttggtactgatcgacgacggttggcaaacattttgccgtgacgacgaaaccgtgagcgacggggggagtttaaattgctctgtgccgggggagcagatgctgaataggttgataaaatttgaagagaatggcaagtttaaggagtataagtgtgggagggagggtaataagggtatgggtgcgtttgtgagggagttgaaggaggaatttagtgggttggagtatgtatatgtgtggcatgcgttttgtgggtactggggaggggttaggcctaaggtgccggggatgccggaggccacggtggttccgaccaagttgtctcccggagcggggangactatgacggaccaggcggtggtgaagatcatggagattggggtggggttggtgccaccgcatcgggcgcatgagttgtacgaggggcttcactctcatctggaatcggtgggaattgatggtgtcaagattgatgtcacgcatattctagagatgctatcggaggaatatggtggtcgtgtcgaactcgctaaagcatattacaaagcactcactgcttccgtgaggaagcatttcaaaggcaatggtgtcatttcaagcatgcagcagtgcaatgatttcatgttccttggtacggaaaccatatcacttggacgagtcgattcattccataaatgtgagttgtggtacattcatgcaggtgatgatttttggtgcacggacccagctggagatccaaacggtacctattggctgcaagggtgtcacatggtgcactgtgcttacaacagcttgtggatgggaaatttcatacacccagattgggacatgttccaatctgatcatgcttgtgccgaattccacgctgcttctagagccatttctggtggaccaatttatgtaagcgactctgttggaaaacacaacttcaagttgcttaagaagcttgttctacctgatggctccattttgcggtgtcaacattatgcacttcccacccgagactgcttatttgtagatcctttacatgatgggaaaacaatgctcaaaatttggaacctcaataaatgttccggggttttgggtctgttcaattgccaaggaggaggttggtgccctgttactaggcgaaacaagagtagctctgactattcacactccgtgacttgctttgcaagtcctcaagacattgaatggggcaaagggaagcacccagtttgcatcaaaggggtggacgtatttgctgtgtacatgtttaaggacgacaagttgaagctgctgaagtacacagagagtgtagaagtttctcttgagccttttagttgtgagcttttgaccgtttctccagtggtgatcttacccagaaaatcaatccaatttgccccaattggattggtaaacatgctcaactctgggggctctattatgtcattggaatttgatcaacaggaaaatttggcgaggattggggtgagaggacatggggaaatgagggtatttgcatcagagaagccagagagtgtcaagattgatggagaatctgtggaatttgattatgttgatagaaccgtgaggctccaagtctcgtggccttgttcttcgaggttgtccgtagtcgagtatttgttctga

SEQ ID NO: 6 - protein, 785 aa, Glycine max
  MOD_RES 355: note = X is encoded by acg, atg, agg, aag, or aug
MAPSLTAKQEAALLNANPHLSIKLQSSTFFANNHPILTQVPPNITTTTPPPHDASTTPAGCFVGFSADEARSRHVISLGKLRGIRFTSIFRFKLWWSTHWSGSNGRDVENETQMMILQNDAVEGRPYVLLLPLLEGPFRASLQPGLHDDVDICMESGSARVTKSRFRTSVYMHVHDDPFTLIDEALKVIRVYLGTFRLMEEKTVPGIIDKFGWCTWDAFYLNVHPEGVREGIKGLVEGGCPPGLVLIDDGWQTFCRDDETVSDGGSLNCSVPGEQMLNRLIKFEENGKFKEYKCGREGNKGMGAFVRELKEEFSGLEYVYVWHAFCGYWGGVRPKVPGMPEATVVPTKLSPGAGXTMTDQAVVKIMEIGVGLVPPHRAHELYEGLHSHLESVGIDGVKIDVTHILEMLSEEYGGRVELAKAYYKALTASVRKHFKGNGVISSMQQCNDFMFLGTETISLGRVDSFHKCELWYIHAGDDFWCTDPAGDPNGTYWLQGCHMVHCAYNSLWMGNFIHPDWDMFQSDHACAEFHAASRAISGGPIYVSDSVGKHNFKLLKKLVLPDGSILRCQHYALPTRDCLFVDPLHDGKTMLKIWNLNKCSGVLGLFNCQGGGWCPVTRRNKSSSDYSHSVTCFASPQDIEWGKGKHPVCIKGVDVFAVYMFKDDKLKLLKYTESVEVSLEPFSCELLTVSPVVILPRKSIQFAPIGLVNMLNSGGSIMSLEFDQQENLARIGVRGHGEMRVFASEKPESVKIDGESVEFDYVDRTVRLQVSWPCSSRLSVVEYLF

SEQ ID NO: 7 - DNA, 34 bp, synthetic construct
  source 1..34: mol_type = other DNA
gcgggcagggcggctggagcaggtgtatatgtgg

SEQ ID NO: 8 - DNA, 26 bp, synthetic construct
  source 1..26: mol_type = other DNA
gcgggctggagcaggtgtatttgcac

SEQ ID NO: 9 - DNA, 23 bp, synthetic construct
  source 1..23: mol_type = other DNA
tgggtctgaccccaccccaatac

SEQ ID NO: 10 - DNA, 20 bp, synthetic construct
  source 1..20: mol_type = other DNA
ctagggccatctctggtgga

SEQ ID NO: 11 - DNA, 20 bp, synthetic construct
  source 1..20: mol_type = other DNA
cgtgtggggagtgcatagtg

SEQ ID NO: 12 - DNA, 42 bp, synthetic construct
  source 1..42: mol_type = other DNA
gcgggcagggcggcatgggtccaagctcgaagaaagcgtcac

SEQ ID NO: 13 - DNA, 34 bp, synthetic construct
  source 1..34: mol_type = other DNA
gcgggcatgggtccaagctcgaagaaagcctcag

SEQ ID NO: 14 - DNA, 27 bp, synthetic construct
  source 1..27: mol_type = other DNA
gagttgcagaggctgaagcccttcatg

SEQ ID NO: 15 - DNA, 20 bp, synthetic construct
  source 1..20: mol_type = other DNA
cactggagttcttggggtgt

SEQ ID NO: 16 - DNA, 20 bp, synthetic construct
  source 1..20: mol_type = other DNA
gcttggctgaaatacgaagc

SEQ ID NO: 17 - DNA, 24 bp, synthetic construct
  source 1..24: mol_type = other DNA
ctgtaacaagatggatgccactac

SEQ ID NO: 18 - DNA, 20 bp, synthetic construct
  source 1..20: mol_type = other DNA
cagtcaaggttagtggacct